European Patent Application EP 4 403 635 A2, published July 24, 2024. Title: FUSION PROTEIN COMPRISING IL-2 PROTEIN AND CD80 PROTEIN AND USE THEREOF. Applicant: GI Innovation, Inc. The sequence listing filed with the application follows.

SEQUENCE LISTING (37 sequences)

SEQ ID NO: 1 - protein, 25 aa, synthetic construct
  REGION 1..25: note = signal peptide (TPA)
MDAMLRGLCCVLLLCGAVFVSPSHA

SEQ ID NO: 2 - protein, 208 aa, synthetic construct [sequence omitted]

SEQ ID NO: 3 - protein, 30 aa, synthetic construct
  REGION 1..30: note = hinge
GSGGGGSGGGGSGGGGSAESKYGPPCPPCP

SEQ ID NO: 4 - protein, 216 aa, synthetic construct
  REGION 1..216: note = immunoglobulin fc
APEAAGGPSVFLFPPKPKDQLMISRTPEVTCVVVDVSQEDPEVQFNWYVDGVEVHNAKTKPREEQFNSTYRVVSVLTVLHQDWLNGKEYKCKVSNKGLPSSIEKTISKAKGQPREPQVYTLPPSQEEMTKNQVSLTCLVKGFYPSDIAVEWESNGQPENNYKTTPPVLDSDGSFFLYSRLTVDKSRWQEGNVFSCSVLHEALHNHYTQKSLSLSLG

SEQ ID NO: 5 - protein, 5 aa, synthetic construct
  REGION 1..5: note = linker
GGGGS

SEQ ID NO: 6 - protein, 133 aa, synthetic construct
  REGION 1..133: note = hIL-2M
APTSSSTKKTQLQLEHLLLDLQMILNGINNYKNPKLTAMLTAKFYMPKKATELKHLQCLEEELKPLEEVLNLAQSKNFHLRPRDLISNINVIVLELKGSETTFMCEYADETATIVEFLNRWITFCQSIISTLT

SEQ ID NO: 7 - protein, 617 aa, synthetic construct
  REGION 1..617: note = fusion protein comprising variants of IL-2 and fragments of CD80
MDAMLRGLCCVLLLCGAVFVSPSHAVIHVTKEVKEVATLSCGHNVSVEELAQTRIYWQKEKKMVLTMMSGDMNIWPEYKNRTIFDITNNLSIVILALRPSDEGTYECVVLKYEKDAFKREHLAEVTLSVKADFPTPSISDFEIPTSNIRRIICSTSGGFPEPHLSWLENGEELNAINTTVSQDPETELYAVSSKLDFNMTTNHSFMCLIKYGHLRVNQTFNWNTTKQEHFPDNGSGGGGSGGGGSGGGGSAESKYGPPCPPCPAPEAAGGPSVFLFPPKPKDQLMISRTPEVTCVVVDVSQEDPEVQFNWYVDGVEVHNAKTKPREEQFNSTYRVVSVLTVLHQDWLNGKEYKCKVSNKGLPSSIEKTISKAKGQPREPQVYTLPPSQEEMTKNQVSLTCLVKGFYPSDIAVEWESNGQPENNYKTTPPVLDSDGSFFLYSRLTVDKSRWQEGNVFSCSVLHEALHNHYTQKSLSLSLGGGGGSAPTSSSTKKTQLQLEHLLLDLQMILNGINNYKNPKLTAMLTAKFYMPKKATELKHLQCLEEELKPLEEVLNLAQSKNFHLRPRDLISNINVIVLELKGSETTFMCEYADETATIVEFLNRWITFCQSIISTLT

SEQ ID NO: 8 - DNA, 1857 bp, synthetic construct
  misc_feature 1..1857: note = nucleotiedes coding fusion protein (GI101)
  source 1..1857: mol_type = other DNA
atggatgctatgctgagaggcctgtgttgcgtgctgctgctgtgtggcgctgtgttcgtgtctccttctcacgctgtgatccacgtgaccaaagaagtgaaagaggtcgccacactgtcctgcggccacaacgtttcagtggaagaactggcccagaccaggatctactggcagaaagaaaagaaaatggtgctgaccatgatgtccggcgacatgaacatctggcctgagtacaagaaccggaccatcttcgacatcaccaacaacctgtccatcgtgattctggccctgaggccttctgatgagggcacctatgagtgcgtggtgctgaagtacgagaaggacgccttcaagcgcgagcacctggctgaagtgacactgtccgtgaaggccgactttcccacaccttccatctccgacttcgagatccctacctccaacatccggcggatcatctgttctacctctggcggctttcctgagcctcacctgtcttggctggaaaacggcgaggaactgaacgccatcaacaccaccgtgtctcaggaccccgaaaccgagctgtacgctgtgtcctccaagctggacttcaacatgaccaccaaccacagcttcatgtgcctgattaagtacggccacctgagagtgaaccagaccttcaactggaacaccaccaagcaagagcacttccctgacaatggatctggcggcggaggttctggcggaggtggaagcggaggcggaggatctgctgagtctaagtatggccctccttgtcctccatgtcctgctccagaagctgctggcggaccctctgtgttcctgtttcctccaaagcctaaggaccagctcatgatctctcggacacccgaagtgacctgcgtggtggtggatgtgtctcaagaggaccctgaggtgcagttcaattggtacgtggacggcgtggaagtgcacaacgccaagaccaagcctagagaggaacagttcaactccacctacagagtggtgtccgtgctgaccgtgctgcaccaggattggctgaacggcaaagagtacaagtgcaaggtgtccaacaagggcctgccttccagcatcgaaaagaccatctccaaggctaagggccagcctagggaaccccaggtttacaccctgcctccaagccaagaggaaatgaccaagaaccaggtgtccctgacctgcctggtcaagggcttctacccttccgacattgccgtggaatgggagtccaatggccagcctgagaacaactacaagaccacacctcctgtgctggactccgacggctccttctttctgtactctcgcctgaccgtggacaagtctagatggcaagagggcaacgtgttctcctgctctgtgctgcacgaggccctgcacaatcactacacccagaagtccctgtctctgtctcttggaggtggtggcggttctgcccctaccagctcctctaccaagaaaacccagctccagttggagcatctgctgctggacctccagatgattctgaacgggatcaacaactataagaaccccaagctgaccgccatgctgaccgctaagttctacatgcccaagaaggccaccgagctgaagcacctccagtgcctggaagaagaactgaagcccctggaagaggtgctgaatctggcccagtccaagaacttccacctgaggccacgggacctgatcagcaacatcaacgtgatcgtgctggaactgaagggctccgagacaacctttatgtgcgagtacgccgacgagacagccaccatcgtggaatttctgaaccggtggatcaccttctgccagagcatcatctccacactgacctgatga

SEQ ID NO: 9 - protein, 592 aa, synthetic construct
  REGION 1..592: note = fusion protein (GI101)
VIHVTKEVKEVATLSCGHNVSVEELAQTRIYWQKEKKMVLTMMSGDMNIWPEYKNRTIFDITNNLSIVILALRPSDEGTYECVVLKYEKDAFKREHLAEVTLSVKADFPTPSISDFEIPTSNIRRIICSTSGGFPEPHLSWLENGEELNAINTTVSQDPETELYAVSSKLDFNMTTNHSFMCLIKYGHLRVNQTFNWNTTKQEHFPDNGSGGGGSGGGGSGGGGSAESKYGPPCPPCPAPEAAGGPSVFLFPPKPKDQLMISRTPEVTCVVVDVSQEDPEVQFNWYVDGVEVHNAKTKPREEQFNSTYRVVSVLTVLHQDWLNGKEYKCKVSNKGLPSSIEKTISKAKGQPREPQVYTLPPSQEEMTKNQVSLTCLVKGFYPSDIAVEWESNGQPENNYKTTPPVLDSDGSFFLYSRLTVDKSRWQEGNVFSCSVLHEALHNHYTQKSLSLSLGGGGGSAPTSSSTKKTQLQLEHLLLDLQMILNGINNYKNPKLTAMLTAKFYMPKKATELKHLQCLEEELKPLEEVLNLAQSKNFHLRPRDLISNINVIVLELKGSETTFMCEYADETATIVEFLNRWITFCQSIISTLT

SEQ ID NO: 10 - protein, 133 aa, synthetic construct [sequence omitted]

SEQ ID NO: 11 - protein, 288 aa, synthetic construct
  REGION 1..288: note = CD80
MGHTRRQGTSPSKCPYLNFFQLLVLAGLSHFCSGVIHVTKEVKEVATLSCGHNVSVEELAQTRIYWQKEKKMVLTMMSGDMNIWPEYKNRTIFDITNNLSIVILALRPSDEGTYECVVLKYEKDAFKREHLAEVTLSVKADFPTPSISDFEIPTSNIRRIICSTSGGFPEPHLSWLENGEELNAINTTVSQDPETELYAVSSKLDFNMTTNHSFMCLIKYGHLRVNQTFNWNTTKQEHFPDNLLPSWAITLISVNGIFVICCLTYCFAPRCRERRRNERLRRESVRPV

SEQ ID NO: 12 - protein, 215 aa, synthetic construct
  REGION 1..215: note = modified Fc
SHTQPLGVFLFPPKPKDTLMISRTPEVTCVVVDVSQEDPEVQFNWYVDGVEVHNAKTKPREEQFNSTYRVVSVLTVLHQDWLNGKEYKCKVSNKGLPSSIEKTISKAKGQPREPQVYTLPPSQEEMTKNQVSLTCLVKGFYPSDIAVEWESNGQPENNYKTTPPVLDSDGSFFLYSRLTVDKSRWQEGNVFSCSVMHEALHNHYTQKSLSLSLGK

SEQ ID NO: 13 - protein, 306 aa, synthetic construct
  REGION 1..306: note = mCD80
MACNCQLMQDTPLLKFPCPRLILLFVLLIRLSQVSSDVDEQLSKSVKDKVLLPCRYNSPHEDESEDRIYWQKHDKVVLSVIAGKLKVWPEYKNRTLYDNTTYSLIILGLVLSDRGTYSCVVQKKERGTYEVKHLALVKLSIKADFSTPNITESGNPSADTKRITCFASGGFPKPRFSWLENGRELPGINTTISQDPESELYTISSQLDFNTTRNHTIKCLIKYGDAHVSEDFTWEKPPEDPPDSKNTLVLFGAGFGAVITVVVIVVIIKCFCKHRSCFRRNEASRETNNSLTFGPEEALAEQTVFL

SEQ ID NO: 14 - DNA, 1848 bp, synthetic construct
  misc_feature 1..1848: note = nucleotiedes coding fusion protein (mGI101)
  source 1..1848: mol_type = other DNA
atggatgctatgctgagaggcctgtgttgcgtgctgctgctgtgtggcgctgtgttcgtgtctccttctcacgctgtggacgagcagctctccaagtccgtgaaggataaggtcctgctgccttgccggtacaactctcctcacgaggacgagtctgaggaccggatctactggcagaaacacgacaaggtggtgctgtccgtgatcgccggaaagctgaaagtgtggcctgagtacaagaacaggaccctgtacgacaacaccacctacagcctgatcatcctgggcctcgtgctgagcgatagaggcacctattcttgcgtggtgcagaagaaagagcggggcacctacgaagtgaagcacctggctctggtcaagctgtccatcaaggccgacttcagcacccctaacatcaccgagtctggcaacccttccgccgacaccaagagaatcacctgtttcgcctctggcggcttccctaagcctcggttctcttggctggaaaacggcagagagctgcccggcatcaataccaccatttctcaggacccagagtccgagctgtacaccatctccagccagctcgactttaacaccaccagaaaccacaccatcaagtgcctgattaagtacggcgacgcccacgtgtccgaggactttacttgggagaaacctcctgaggaccctcctgactctggatctggcggcggaggttctggcggaggtggaagcggaggcggaggatctgctgagtctaagtatggccctccttgtcctccatgtcctgctccagaagctgctggcggaccctctgtgttcctgtttcctccaaagcctaaggaccagctcatgatctctcggacccctgaagtgacctgcgtggtggtggatgtgtctcaagaggaccctgaggtgcagttcaattggtacgtggacggcgtggaagtgcacaacgccaagaccaagcctagagaggaacagttcaactccacctatagagtggtgtccgtgctgaccgtgctgcaccaggattggctgaacggcaaagagtacaagtgcaaggtgtccaacaagggcctgccttccagcatcgaaaagaccatcagcaaggctaagggccagcctagggaaccccaggtttacaccctgcctccaagccaagaggaaatgaccaagaaccaggtgtccctgacctgcctggtcaagggcttctacccttccgacattgccgtggaatgggagtccaatggccagcctgagaacaactacaagaccacacctcctgtgctggactccgacggctccttctttctgtactctcgcctgaccgtggacaagtctaggtggcaagagggcaacgtgttctcctgctctgtgctgcacgaggctctgcacaaccactacacccagaagtccctgtctctgtctcttggaggtggtggcggttctgcccctacctccagctctaccaagaaaacccagctccagttggagcatctgctgctggacctccagatgatcctgaatggcatcaacaattacaagaaccccaagctgaccgccatgctgaccgctaagttctacatgcccaagaaggccaccgagctgaagcacttgcagtgcctggaagaggaactgaagcccctggaagaagtgctgaatctggcccagtccaagaacttccacctgaggcctagggacctgatctccaacatcaacgtgatcgtgctggaactgaaaggctccgagacaaccttcatgtgcgagtacgccgacgagacagccaccatcgtggaatttctgaaccggtggatcaccttctgccagagcatcatctccacactgacc

SEQ ID NO: 15 - protein, 616 aa, synthetic construct
  REGION 1..616: note = fusion protein (mGI101)
MDAMLRGLCCVLLLCGAVFVSPSHAVDEQLSKSVKDKVLLPCRYNSPHEDESEDRIYWQKHDKVVLSVIAGKLKVWPEYKNRTLYDNTTYSLIILGLVLSDRGTYSCVVQKKERGTYEVKHLALVKLSIKADFSTPNITESGNPSADTKRITCFASGGFPKPRFSWLENGRELPGINTTISQDPESELYTISSQLDFNTTRNHTIKCLIKYGDAHVSEDFTWEKPPEDPPDSGSGGGGSGGGGSGGGGSAESKYGPPCPPCPAPEAAGGPSVFLFPPKPKDQLMISRTPEVTCVVVDVSQEDPEVQFNWYVDGVEVHNAKTKPREEQFNSTYRVVSVLTVLHQDWLNGKEYKCKVSNKGLPSSIEKTISKAKGQPREPQVYTLPPSQEEMTKNQVSLTCLVKGFYPSDIAVEWESNGQPENNYKTTPPVLDSDGSFFLYSRLTVDKSRWQEGNVFSCSVLHEALHNHYTQKSLSLSLGGGGGSAPTSSSTKKTQLQLEHLLLDLQMILNGINNYKNPKLTAMLTAKFYMPKKATELKHLQCLEEELKPLEEVLNLAQSKNFHLRPRDLISNINVIVLELKGSETTFMCEYADETATIVEFLNRWITFCQSIISTLT

SEQ ID NO: 16 - DNA, 1437 bp, synthetic construct
  misc_feature 1..1437: note = nucleotiedes coding fusion protein (GI101C1)
  source 1..1437: mol_type = other DNA
atggatgctatgctgagaggcctgtgttgcgtgctgctgctgtgtggcgctgtgttcgtgtctccttctcacgctgtgatccacgtgaccaaagaagtgaaagaggtcgccacactgtcctgcggccacaacgtttcagtggaagaactggcccagaccaggatctactggcagaaagaaaagaaaatggtgctgaccatgatgtccggcgacatgaacatctggcctgagtacaagaaccggaccatcttcgacatcaccaacaacctgtccatcgtgattctggccctgaggccttctgatgagggcacctatgagtgcgtggtgctgaagtacgagaaggacgccttcaagcgcgagcacctggctgaagtgacactgtccgtgaaggccgactttcccacaccttccatctccgacttcgagatccctacctccaacatccggcggatcatctgttctacctctggcggctttcctgagcctcacctgtcttggctggaaaacggcgaggaactgaacgccatcaacaccaccgtgtctcaggaccccgaaaccgagctgtacgctgtgtcctccaagctggacttcaacatgaccaccaaccacagcttcatgtgcctgattaagtacggccacctgagagtgaaccagaccttcaactggaacaccaccaagcaagagcacttccctgacaatggatctggcggcggaggttctggcggaggtggaagcggaggcggaggatctgctgagtctaagtatggccctccttgtcctccatgtcctgctccagaagctgctggcggaccctctgtgttcctgtttcctccaaagcctaaggaccagctcatgatctctcggacacccgaagtgacctgcgtggtggtggatgtgtctcaagaggaccctgaggtgcagttcaattggtacgtggacggcgtggaagtgcacaacgccaagaccaagcctagagaggaacagttcaactccacctacagagtggtgtccgtgctgaccgtgctgcaccaggattggctgaacggcaaagagtacaagtgcaaggtgtccaacaagggcctgccttccagcatcgaaaagaccatctccaaggctaagggccagcctagggaaccccaggtttacaccctgcctccaagccaagaggaaatgaccaagaaccaggtgtccctgacctgcctggtcaagggcttctacccttccgacattgccgtggaatgggagtccaatggccagcctgagaacaactacaagaccacacctcctgtgctggactccgacggctccttctttctgtactctcgcctgaccgtggacaagtctaggtggcaagagggcaacgtgttctcctgctctgtgctgcacgaggccctgcacaatcactacacccagaagtccctgtctctgtccctgggc

SEQ ID NO: 17 - protein, 454 aa, synthetic construct
  REGION 1..454: note = fusion protein (GI101C1)
VIHVTKEVKEVATLSCGHNVSVEELAQTRIYWQKEKKMVLTMMSGDMNIWPEYKNRTIFDITNNLSIVILALRPSDEGTYECVVLKYEKDAFKREHLAEVTLSVKADFPTPSISDFEIPTSNIRRIICSTSGGFPEPHLSWLENGEELNAINTTVSQDPETELYAVSSKLDFNMTTNHSFMCLIKYGHLRVNQTFNWNTTKQEHFPDNGSGGGGSGGGGSGGGGSAESKYGPPCPPCPAPEAAGGPSVFLFPPKPKDQLMISRTPEVTCVVVDVSQEDPEVQFNWYVDGVEVHNAKTKPREEQFNSTYRVVSVLTVLHQDWLNGKEYKCKVSNKGLPSSIEKTISKAKGQPREPQVYTLPPSQEEMTKNQVSLTCLVKGFYPSDIAVEWESNGQPENNYKTTPPVLDSDGSFFLYSRLTVDKSRWQEGNVFSCSVLHEALHNHYTQKSLSLSLG

SEQ ID NO: 18 - DNA, 1176 bp, synthetic construct
  misc_feature 1..1176: note = nucleotiedes coding fusion protein (GI101C2)
  source 1..1176: mol_type = other DNA
atggatgctatgctgagaggcctgtgttgcgtgctgctgctgtgtggcgctgtgttcgtgtctccatctcacgccgctgagtctaagtacggccctccttgtcctccatgtcctgctccagaagctgctggcggaccctctgtgttcctgtttcctccaaagcctaaggaccagctcatgatctctcggacccctgaagtgacctgcgtggtggtggatgtgtctcaagaggaccctgaggtgcagttcaattggtacgtggacggcgtggaagtgcacaacgccaagaccaagcctagagaggaacagttcaactccacctacagagtggtgtccgtgctgaccgtgctgcaccaggattggctgaacggcaaagagtacaagtgcaaggtgtccaacaagggcctgccttccagcatcgaaaagaccatctccaaggctaagggccagcctagggaaccccaggtttacaccctgcctccaagccaagaggaaatgaccaagaaccaggtgtccctgacctgcctggtcaagggcttctacccttccgacattgccgtggaatgggagtccaatggccagcctgagaacaactacaagaccacacctcctgtgctggactccgacggctccttctttctgtactctcgcctgaccgtggacaagtctaggtggcaagagggcaacgtgttctcctgctctgtgctgcacgaggccctgcacaatcactacacccagaagtccctgtctctgtctcttggcggaggcggaggatctgctcctacctccagctccaccaagaaaacccagctccagttggagcatctgctgctggacctccagatgatcctgaatggcatcaacaattacaagaaccccaagctgaccgccatgctgaccgctaagttctacatgcccaagaaggccaccgagctgaagcacctccagtgcctggaagaggaactgaagcccctggaagaagtgctgaatctggcccagtccaagaacttccacctgaggcctagggacctgatctccaacatcaacgtgatcgtgctggaactgaaaggctccgagacaaccttcatgtgcgagtacgccgacgagacagccaccatcgtggaatttctgaaccggtggatcaccttctgccagtccatcatctccacactgacc

SEQ ID NO: 19 - protein, 367 aa, synthetic construct
  REGION 1..367: note = fusion protein (GI101C2)
AESKYGPPCPPCPAPEAAGGPSVFLFPPKPKDQLMISRTPEVTCVVVDVSQEDPEVQFNWYVDGVEVHNAKTKPREEQFNSTYRVVSVLTVLHQDWLNGKEYKCKVSNKGLPSSIEKTISKAKGQPREPQVYTLPPSQEEMTKNQVSLTCLVKGFYPSDIAVEWESNGQPENNYKTTPPVLDSDGSFFLYSRLTVDKSRWQEGNVFSCSVLHEALHNHYTQKSLSLSLGGGGGSAPTSSSTKKTQLQLEHLLLDLQMILNGINNYKNPKLTAMLTAKFYMPKKATELKHLQCLEEELKPLEEVLNLAQSKNFHLRPRDLISNINVIVLELKGSETTFMCEYADETATIVEFLNRWITFCQSIISTLT

SEQ ID NO: 20 - DNA, 1434 bp, synthetic construct
  misc_feature 1..1434: note = nucleotiedes coding fusion protein (mGI101C1)
  source 1..1434: mol_type = other DNA
atggatgctatgctgagaggcctgtgttgcgtgctgctgctgtgtggcgctgtgttcgtgtctccttctcacgctgtggacgagcagctctccaagtccgtgaaggataaggtcctgctgccttgccggtacaactctcctcacgaggacgagtctgaggaccggatctactggcagaaacacgacaaggtggtgctgtccgtgatcgccggaaagctgaaagtgtggcctgagtacaagaacaggaccctgtacgacaacaccacctacagcctgatcatcctgggcctcgtgctgagcgatagaggcacctattcttgcgtggtgcagaagaaagagcggggcacctacgaagtgaagcacctggctctggtcaagctgtccatcaaggccgacttcagcacccctaacatcaccgagtctggcaacccttccgccgacaccaagagaatcacctgtttcgcctctggcggcttccctaagcctcggttctcttggctggaaaacggcagagagctgcccggcatcaataccaccatttctcaggacccagagtccgagctgtacaccatctccagccagctcgactttaacaccaccagaaaccacaccatcaagtgcctgattaagtacggcgacgcccacgtgtccgaggactttacttgggagaaacctcctgaggaccctcctgactctggatctggcggcggaggttctggcggaggtggaagcggaggcggaggatctgctgagtctaagtatggccctccttgtcctccatgtcctgctccagaagctgctggcggaccctctgtgttcctgtttcctccaaagcctaaggaccagctcatgatctctcggacccctgaagtgacctgcgtggtggtggatgtgtctcaagaggaccctgaggtgcagttcaattggtacgtggacggcgtggaagtgcacaacgccaagaccaagcctagagaggaacagttcaactccacctatagagtggtgtccgtgctgaccgtgctgcaccaggattggctgaacggcaaagagtacaagtgcaaggtgtccaacaagggcctgccttccagcatcgaaaagaccatcagcaaggctaagggccagcctagggaaccccaggtttacaccctgcctccaagccaagaggaaatgaccaagaaccaggtgtccctgacctgcctggtcaagggcttctacccttccgacattgccgtggaatgggagtccaatggccagcctgagaacaactacaagaccacacctcctgtgctggactccgacggctccttctttctgtactctcgcctgaccgtggacaagtctaggtggcaagagggcaacgtgttctcctgctctgtgctgcacgaggctctgcacaaccactacacccagaagtccctgtctctgtccctgggc

SEQ ID NO: 21 - protein, 478 aa, synthetic construct
  REGION 1..478: note = fusion protein (mGI101C1)
MDAMLRGLCCVLLLCGAVFVSPSHAVDEQLSKSVKDKVLLPCRYNSPHEDESEDRIYWQKHDKVVLSVIAGKLKVWPEYKNRTLYDNTTYSLIILGLVLSDRGTYSCVVQKKERGTYEVKHLALVKLSIKADFSTPNITESGNPSADTKRITCFASGGFPKPRFSWLENGRELPGINTTISQDPESELYTISSQLDFNTTRNHTIKCLIKYGDAHVSEDFTWEKPPEDPPDSGSGGGGSGGGGSGGGGSAESKYGPPCPPCPAPEAAGGPSVFLFPPKPKDQLMISRTPEVTCVVVDVSQEDPEVQFNWYVDGVEVHNAKTKPREEQFNSTYRVVSVLTVLHQDWLNGKEYKCKVSNKGLPSSIEKTISKAKGQPREPQVYTLPPSQEEMTKNQVSLTCLVKGFYPSDIAVEWESNGQPENNYKTTPPVLDSDGSFFLYSRLTVDKSRWQEGNVFSCSVLHEALHNHYTQKSLSLSLG

SEQ ID NO: 22 - protein, 133 aa, synthetic construct
  REGION 1..133: note = variants of IL-2 (3M, M45)
APTSSSTKKTQLQLEHLLLDLQMILNGINNYKNPKLTAMLTAKFAMPKKATELKHLQCLEEELKPLEEVLNLAQSKNFHLRPRDLISNINVIVLELKGSETTFMCEYADETATIVEFLNRWITFCQSIISTLT

SEQ ID NO: 23 - protein, 133 aa, synthetic construct
  REGION 1..133: note = variants of IL-2 (3M, M61)
APTSSSTKKTQLQLEHLLLDLQMILNGINNYKNPKLTAMLTAKFYMPKKATELKHLQCLERELKPLEEVLNLAQSKNFHLRPRDLISNINVIVLELKGSETTFMCEYADETATIVEFLNRWITFCQSIISTLT

SEQ ID NO: 24 - protein, 133 aa, synthetic construct
  REGION 1..133: note = variants of IL-2 (3M, M72)
APTSSSTKKTQLQLEHLLLDLQMILNGINNYKNPKLTAMLTAKFYMPKKATELKHLQCLEEELKPLEEVLNGAQSKNFHLRPRDLISNINVIVLELKGSETTFMCEYADETATIVEFLNRWITFCQSIISTLT

SEQ ID NO: 25 - DNA, 1851 bp, synthetic construct
  misc_feature 1..1851: note = nucleotiedes coding fusion protein (GI102-M45)
  source 1..1851: mol_type = other DNA
atggatgctatgctgagaggcctgtgttgcgtgctgctgctgtgtggcgctgtgttcgtgtctccttctcacgctgtgatccacgtgaccaaagaagtgaaagaggtcgccacactgtcctgcggccacaacgtttcagtggaagaactggcccagaccaggatctactggcagaaagaaaagaaaatggtgctgaccatgatgtccggcgacatgaacatctggcctgagtacaagaaccggaccatcttcgacatcaccaacaacctgtccatcgtgattctggccctgaggccttctgatgagggcacctatgagtgcgtggtgctgaagtacgagaaggacgccttcaagcgcgagcacctggctgaagtgacactgtccgtgaaggccgactttcccacaccttccatctccgacttcgagatccctacctccaacatccggcggatcatctgttctacctctggcggctttcctgagcctcacctgtcttggctggaaaacggcgaggaactgaacgccatcaacaccaccgtgtctcaggaccccgaaaccgagctgtacgctgtgtcctccaagctggacttcaacatgaccaccaaccacagcttcatgtgcctgattaagtacggccacctgagagtgaaccagaccttcaactggaacaccaccaagcaagagcacttccctgacaatggatctggcggcggaggttctggcggaggtggaagcggaggcggaggatctgctgagtctaagtatggccctccttgtcctccatgtcctgctccagaagctgctggcggaccctctgtgttcctgtttcctccaaagcctaaggaccagctcatgatctctcggacacccgaagtgacctgcgtggtggtggatgtgtctcaagaggaccctgaggtgcagttcaattggtacgtggacggcgtggaagtgcacaacgccaagaccaagcctagagaggaacagttcaactccacctacagagtggtgtccgtgctgaccgtgctgcaccaggattggctgaacggcaaagagtacaagtgcaaggtgtccaacaagggcctgccttccagcatcgaaaagaccatctccaaggctaagggccagcctagggaaccccaggtttacaccctgcctccaagccaagaggaaatgaccaagaaccaggtgtccctgacctgcctggtcaagggcttctacccttccgacattgccgtggaatgggagtccaatggccagcctgagaacaactacaagaccacacctcctgtgctggactccgacggctccttctttctgtactctcgcctgaccgtggacaagtctagatggcaagagggcaacgtgttctcctgctctgtgctgcacgaggccctgcacaatcactacacccagaagtccctgtctctgtctcttggaggtggtggcggttctgcccctaccagctcctctaccaagaaaacccagctccagttggagcatctgctgctggacctccagatgattctgaacgggatcaacaactataagaaccccaagctgaccgccatgctgaccgctaagttcgccatgcccaagaaggccaccgagctgaagcacctccagtgcctggaagaagaactgaagcccctggaagaggtgctgaatctggcccagtccaagaacttccacctgaggccacgggacctgatcagcaacatcaacgtgatcgtgctggaactgaagggctccgagacaacctttatgtgcgagtacgccgacgagacagccaccatcgtggaatttctgaaccggtggatcaccttctgccagagcatcatctccacactgacc

SEQ ID NO: 26 - protein, 592 aa, synthetic construct
  REGION 1..592: note = fusion protein (GI102-M45)
VIHVTKEVKEVATLSCGHNVSVEELAQTRIYWQKEKKMVLTMMSGDMNIWPEYKNRTIFDITNNLSIVILALRPSDEGTYECVVLKYEKDAFKREHLAEVTLSVKADFPTPSISDFEIPTSNIRRIICSTSGGFPEPHLSWLENGEELNAINTTVSQDPETELYAVSSKLDFNMTTNHSFMCLIKYGHLRVNQTFNWNTTKQEHFPDNGSGGGGSGGGGSGGGGSAESKYGPPCPPCPAPEAAGGPSVFLFPPKPKDQLMISRTPEVTCVVVDVSQEDPEVQFNWYVDGVEVHNAKTKPREEQFNSTYRVVSVLTVLHQDWLNGKEYKCKVSNKGLPSSIEKTISKAKGQPREPQVYTLPPSQEEMTKNQVSLTCLVKGFYPSDIAVEWESNGQPENNYKTTPPVLDSDGSFFLYSRLTVDKSRWQEGNVFSCSVLHEALHNHYTQKSLSLSLGGGGGSAPTSSSTKKTQLQLEHLLLDLQMILNGINNYKNPKLTAMLTAKFAMPKKATELKHLQCLEEELKPLEEVLNLAQSKNFHLRPRDLISNINVIVLELKGSETTFMCEYADETATIVEFLNRWITFCQSIISTLT

SEQ ID NO: 27 - DNA, 1851 bp, synthetic construct
  misc_feature 1..1851: note = nucleotiedes coding fusion protein (GI102-M61)
  source 1..1851: mol_type = other DNA
atggatgctatgctgagaggcctgtgttgcgtgctgctgctgtgtggcgctgtgttcgtgtctccttctcacgctgtgatccacgtgaccaaagaagtgaaagaggtcgccacactgtcctgcggccacaacgtttcagtggaagaactggcccagaccaggatctactggcagaaagaaaagaaaatggtgctgaccatgatgtccggcgacatgaacatctggcctgagtacaagaaccggaccatcttcgacatcaccaacaacctgtccatcgtgattctggccctgaggccttctgatgagggcacctatgagtgcgtggtgctgaagtacgagaaggacgccttcaagcgcgagcacctggctgaagtgacactgtccgtgaaggccgactttcccacaccttccatctccgacttcgagatccctacctccaacatccggcggatcatctgttctacctctggcggctttcctgagcctcacctgtcttggctggaaaacggcgaggaactgaacgccatcaacaccaccgtgtctcaggaccccgaaaccgagctgtacgctgtgtcctccaagctggacttcaacatgaccaccaaccacagcttcatgtgcctgattaagtacggccacctgagagtgaaccagaccttcaactggaacaccaccaagcaagagcacttccctgacaatggatctggcggcggaggttctggcggaggtggaagcggaggcggaggatctgctgagtctaagtatggccctccttgtcctccatgtcctgctccagaagctgctggcggaccctctgtgttcctgtttcctccaaagcctaaggaccagctcatgatctctcggacacccgaagtgacctgcgtggtggtggatgtgtctcaagaggaccctgaggtgcagttcaattggtacgtggacggcgtggaagtgcacaacgccaagaccaagcctagagaggaacagttcaactccacctacagagtggtgtccgtgctgaccgtgctgcaccaggattggctgaacggcaaagagtacaagtgcaaggtgtccaacaagggcctgccttccagcatcgaaaagaccatctccaaggctaagggccagcctagggaaccccaggtttacaccctgcctccaagccaagaggaaatgaccaagaaccaggtgtccctgacctgcctggtcaagggcttctacccttccgacattgccgtggaatgggagtccaatggccagcctgagaacaactacaagaccacacctcctgtgctggactccgacggctccttctttctgtactctcgcctgaccgtggacaagtctagatggcaagagggcaacgtgttctcctgctctgtgctgcacgaggccctgcacaatcactacacccagaagtccctgtctctgtctcttggaggtggtggcggttctgcccctaccagctcctctaccaagaaaacccagctccagttggagcatctgctgctggacctccagatgattctgaacgggatcaacaactataagaaccccaagctgaccgccatgctgaccgctaagttctacatgcccaagaaggccaccgagctgaagcacctccagtgcctggaaagggaactgaagcccctggaagaggtgctgaatctggcccagtccaagaacttccacctgaggccacgggacctgatcagcaacatcaacgtgatcgtgctggaactgaagggctccgagacaacctttatgtgcgagtacgccgacgagacagccaccatcgtggaatttctgaaccggtggatcaccttctgccagagcatcatctccacactgacc

SEQ ID NO: 28 - protein, 592 aa, synthetic construct
  REGION 1..592: note = fusion protein (GI102-M61)
VIHVTKEVKEVATLSCGHNVSVEELAQTRIYWQKEKKMVLTMMSGDMNIWPEYKNRTIFDITNNLSIVILALRPSDEGTYECVVLKYEKDAFKREHLAEVTLSVKADFPTPSISDFEIPTSNIRRIICSTSGGFPEPHLSWLENGEELNAINTTVSQDPETELYAVSSKLDFNMTTNHSFMCLIKYGHLRVNQTFNWNTTKQEHFPDNGSGGGGSGGGGSGGGGSAESKYGPPCPPCPAPEAAGGPSVFLFPPKPKDQLMISRTPEVTCVVVDVSQEDPEVQFNWYVDGVEVHNAKTKPREEQFNSTYRVVSVLTVLHQDWLNGKEYKCKVSNKGLPSSIEKTISKAKGQPREPQVYTLPPSQEEMTKNQVSLTCLVKGFYPSDIAVEWESNGQPENNYKTTPPVLDSDGSFFLYSRLTVDKSRWQEGNVFSCSVLHEALHNHYTQKSLSLSLGGGGGSAPTSSSTKKTQLQLEHLLLDLQMILNGINNYKNPKLTAMLTAKFYMPKKATELKHLQCLERELKPLEEVLNLAQSKNFHLRPRDLISNINVIVLELKGSETTFMCEYADETATIVEFLNRWITFCQSIISTLT

SEQ ID NO: 29 - DNA, 1857 bp, synthetic construct
  misc_feature 1..1857: note = nucleotiedes coding fusion protein (GI102-M72)
  source 1..1857: mol_type = other DNA
atggatgctatgctgagaggcctgtgttgcgtgctgctgctgtgtggcgctgtgttcgtgtctccttctcacgctgtgatccacgtgaccaaagaagtgaaagaggtcgccacactgtcctgcggccacaacgtttcagtggaagaactggcccagaccaggatctactggcagaaagaaaagaaaatggtgctgaccatgatgtccggcgacatgaacatctggcctgagtacaagaaccggaccatcttcgacatcaccaacaacctgtccatcgtgattctggccctgaggccttctgatgagggcacctatgagtgcgtggtgctgaagtacgagaaggacgccttcaagcgcgagcacctggctgaagtgacactgtccgtgaaggccgactttcccacaccttccatctccgacttcgagatccctacctccaacatccggcggatcatctgttctacctctggcggctttcctgagcctcacctgtcttggctggaaaacggcgaggaactgaacgccatcaacaccaccgtgtctcaggaccccgaaaccgagctgtacgctgtgtcctccaagctggacttcaacatgaccaccaaccacagcttcatgtgcctgattaagtacggccacctgagagtgaaccagaccttcaactggaacaccaccaagcaagagcacttccctgacaatggatctggcggcggaggttctggcggaggtggaagcggaggcggaggatctgctgagtctaagtatggccctccttgtcctccatgtcctgctccagaagctgctggcggaccctctgtgttcctgtttcctccaaagcctaaggaccagctcatgatctctcggacacccgaagtgacctgcgtggtggtggatgtgtctcaagaggaccctgaggtgcagttcaattggtacgtggacggcgtggaagtgcacaacgccaagaccaagcctagagaggaacagttcaactccacctacagagtggtgtccgtgctgaccgtgctgcaccaggattggctgaacggcaaagagtacaagtgcaaggtgtccaacaagggcctgccttccagcatcgaaaagaccatctccaaggctaagggccagcctagggaaccccaggtttacaccctgcctccaagccaagaggaaatgaccaagaaccaggtgtccctgacctgcctggtcaagggcttctacccttccgacattgccgtggaatgggagtccaatggccagcctgagaacaactacaagaccacacctcctgtgctggactccgacggctccttctttctgtactctcgcctgaccgtggacaagtctagatggcaagagggcaacgtgttctcctgctctgtgctgcacgaggccctgcacaatcactacacccagaagtccctgtctctgtctcttggaggtggtggcggttctgcccctaccagctcctctaccaagaaaacccagctccagttggagcatctgctgctggacctccagatgattctgaacgggatcaacaactataagaaccccaagctgaccgccatgctgaccgctaagttctacatgcccaagaaggccaccgagctgaagcacctccagtgcctggaagaagaactgaagcccctggaagaggtgctgaatggggcccagtccaagaacttccacctgaggccacgggacctgatcagcaacatcaacgtgatcgtgctggaactgaagggctccgagacaacctttatgtgcgagtacgccgacgagacagccaccatcgtggaatttctgaaccggtggatcaccttctgccagagcatcatctccacactgacctgatga

SEQ ID NO: 30 - protein, 592 aa, synthetic construct
  REGION 1..592: note = fusion protein (GI102-M72)
VIHVTKEVKEVATLSCGHNVSVEELAQTRIYWQKEKKMVLTMMSGDMNIWPEYKNRTIFDITNNLSIVILALRPSDEGTYECVVLKYEKDAFKREHLAEVTLSVKADFPTPSISDFEIPTSNIRRIICSTSGGFPEPHLSWLENGEELNAINTTVSQDPETELYAVSSKLDFNMTTNHSFMCLIKYGHLRVNQTFNWNTTKQEHFPDNGSGGGGSGGGGSGGGGSAESKYGPPCPPCPAPEAAGGPSVFLFPPKPKDQLMISRTPEVTCVVVDVSQEDPEVQFNWYVDGVEVHNAKTKPREEQFNSTYRVVSVLTVLHQDWLNGKEYKCKVSNKGLPSSIEKTISKAKGQPREPQVYTLPPSQEEMTKNQVSLTCLVKGFYPSDIAVEWESNGQPENNYKTTPPVLDSDGSFFLYSRLTVDKSRWQEGNVFSCSVLHEALHNHYTQKSLSLSLGGGGGSAPTSSSTKKTQLQLEHLLLDLQMILNGINNYKNPKLTAMLTAKFYMPKKATELKHLQCLEEELKPLEEVLNGAQSKNFHLRPRDLISNINVIVLELKGSETTFMCEYADETATIVEFLNRWITFCQSIISTLT

SEQ ID NO: 31 - DNA, 1851 bp, synthetic construct
  misc_feature 1..1851: note = nucleotiedes coding fusion protein (GI101w)
  source 1..1851: mol_type = other DNA
atggatgctatgctgagaggcctgtgttgcgtgctgctgctgtgtggcgctgtgttcgtgtctccttctcacgctgtgatccacgtgaccaaagaagtgaaagaggtcgccacactgtcctgcggccacaacgtttcagtggaagaactggcccagaccaggatctactggcagaaagaaaagaaaatggtgctgaccatgatgtccggcgacatgaacatctggcctgagtacaagaaccggaccatcttcgacatcaccaacaacctgtccatcgtgattctggccctgaggccttctgatgagggcacctatgagtgcgtggtgctgaagtacgagaaggacgccttcaagcgcgagcacctggctgaagtgacactgtccgtgaaggccgactttcccacaccttccatctccgacttcgagatccctacctccaacatccggcggatcatctgttctacctctggcggctttcctgagcctcacctgtcttggctggaaaacggcgaggaactgaacgccatcaacaccaccgtgtctcaggaccccgaaaccgagctgtacgctgtgtcctccaagctggacttcaacatgaccaccaaccacagcttcatgtgcctgattaagtacggccacctgagagtgaaccagaccttcaactggaacaccaccaagcaagagcacttccctgacaatggatctggcggcggaggttctggcggaggtggaagcggaggcggaggatctgctgagtctaagtatggccctccttgtcctccatgtcctgctccagaagctgctggcggaccctctgtgttcctgtttcctccaaagcctaaggaccagctcatgatctctcggacacccgaagtgacctgcgtggtggtggatgtgtctcaagaggaccctgaggtgcagttcaattggtacgtggacggcgtggaagtgcacaacgccaagaccaagcctagagaggaacagttcaactccacctacagagtggtgtccgtgctgaccgtgctgcaccaggattggctgaacggcaaagagtacaagtgcaaggtgtccaacaagggcctgccttccagcatcgaaaagaccatctccaaggctaagggccagcctagggaaccccaggtttacaccctgcctccaagccaagaggaaatgaccaagaaccaggtgtccctgacctgcctggtcaagggcttctacccttccgacattgccgtggaatgggagtccaatggccagcctgagaacaactacaagaccacacctcctgtgctggactccgacggctccttctttctgtactctcgcctgaccgtggacaagtctagatggcaagagggcaacgtgttctcctgctctgtgctgcacgaggccctgcacaatcactacacccagaagtccctgtctctgtctcttggaggtggtggcggttctgcccctaccagctcctctaccaagaaaacccagctccagttggagcatctgctgctggacctccagatgattctgaacgggatcaacaactataagaaccccaagctgacccgcatgctgacctttaagttctacatgcccaagaaggccaccgagctgaagcacctccagtgcctggaagaagaactgaagcccctggaagaggtgctgaatctggcccagtccaagaacttccacctgaggccacgggacctgatcagcaacatcaacgtgatcgtgctggaactgaagggctccgagacaacctttatgtgcgagtacgccgacgagacagccaccatcgtggaatttctgaaccggtggatcaccttctgccagagcatcatctccacactgacc

SEQ ID NO: 32 - protein, 592 aa, synthetic construct
  REGION 1..592: note = fusion protein (GI101w)
VIHVTKEVKEVATLSCGHNVSVEELAQTRIYWQKEKKMVLTMMSGDMNIWPEYKNRTIFDITNNLSIVILALRPSDEGTYECVVLKYEKDAFKREHLAEVTLSVKADFPTPSISDFEIPTSNIRRIICSTSGGFPEPHLSWLENGEELNAINTTVSQDPETELYAVSSKLDFNMTTNHSFMCLIKYGHLRVNQTFNWNTTKQEHFPDNGSGGGGSGGGGSGGGGSAESKYGPPCPPCPAPEAAGGPSVFLFPPKPKDQLMISRTPEVTCVVVDVSQEDPEVQFNWYVDGVEVHNAKTKPREEQFNSTYRVVSVLTVLHQDWLNGKEYKCKVSNKGLPSSIEKTISKAKGQPREPQVYTLPPSQEEMTKNQVSLTCLVKGFYPSDIAVEWESNGQPENNYKTTPPVLDSDGSFFLYSRLTVDKSRWQEGNVFSCSVLHEALHNHYTQKSLSLSLGGGGGSAPTSSSTKKTQLQLEHLLLDLQMILNGINNYKNPKLTRMLTFKFYMPKKATELKHLQCLEEELKPLEEVLNLAQSKNFHLRPRDLISNINVIVLELKGSETTFMCEYADETATIVEFLNRWITFCQSIISTLT

SEQ ID NO: 33 - DNA, 1848 bp, synthetic construct
  misc_feature 1..1848: note = nucleotiedes coding fusion protein (mGI102-M61)
  source 1..1848: mol_type = other DNA
atggatgctatgctgagaggcctgtgttgcgtgctgctgctgtgtggcgctgtgttcgtgtctccttctcacgctgtggacgagcagctctccaagtccgtgaaggataaggtcctgctgccttgccggtacaactctcctcacgaggacgagtctgaggaccggatctactggcagaaacacgacaaggtggtgctgtccgtgatcgccggaaagctgaaagtgtggcctgagtacaagaacaggaccctgtacgacaacaccacctacagcctgatcatcctgggcctcgtgctgagcgatagaggcacctattcttgcgtggtgcagaagaaagagcggggcacctacgaagtgaagcacctggctctggtcaagctgtccatcaaggccgacttcagcacccctaacatcaccgagtctggcaacccttccgccgacaccaagagaatcacctgtttcgcctctggcggcttccctaagcctcggttctcttggctggaaaacggcagagagctgcccggcatcaataccaccatttctcaggacccagagtccgagctgtacaccatctccagccagctcgactttaacaccaccagaaaccacaccatcaagtgcctgattaagtacggcgacgcccacgtgtccgaggactttacttgggagaaacctcctgaggaccctcctgactctggatctggcggcggaggttctggcggaggtggaagcggaggcggaggatctgctgagtctaagtatggccctccttgtcctccatgtcctgctccagaagctgctggcggaccctctgtgttcctgtttcctccaaagcctaaggaccagctcatgatctctcggacccctgaagtgacctgcgtggtggtggatgtgtctcaagaggaccctgaggtgcagttcaattggtacgtggacggcgtggaagtgcacaacgccaagaccaagcctagagaggaacagttcaactccacctatagagtggtgtccgtgctgaccgtgctgcaccaggattggctgaacggcaaagagtacaagtgcaaggtgtccaacaagggcctgccttccagcatcgaaaagaccatcagcaaggctaagggccagcctagggaaccccaggtttacaccctgcctccaagccaagaggaaatgaccaagaaccaggtgtccctgacctgcctggtcaagggcttctacccttccgacattgccgtggaatgggagtccaatggccagcctgagaacaactacaagaccacacctcctgtgctggactccgacggctccttctttctgtactctcgcctgaccgtggacaagtctaggtggcaagagggcaacgtgttctcctgctctgtgctgcacgaggctctgcacaaccactacacccagaagtccctgtctctgtctcttggaggtggtggcggttctgcccctacctccagctctaccaagaaaacccagctccagttggagcatctgctgctggacctccagatgatcctgaatggcatcaacaattacaagaaccccaagctgaccgccatgctgaccgctaagttctacatgcccaagaaggccaccgagctgaagcacttgcagtgcctggaaagggaactgaagcccctggaagaagtgctgaatctggcccagtccaagaacttccacctgaggcctagggacctgatctccaacatcaacgtgatcgtgctggaactgaaaggctccgagacaaccttcatgtgcgagtacgccgacgagacagccaccatcgtggaatttctgaaccggtggatcaccttctgccagagcatcatctccacactgacc

SEQ ID NO: 34 - protein, 616 aa, synthetic construct
  REGION 1..616: note = fusion protein (mGI102-M61)
MDAMLRGLCCVLLLCGAVFVSPSHAVDEQLSKSVKDKVLLPCRYNSPHEDESEDRIYWQKHDKVVLSVIAGKLKVWPEYKNRTLYDNTTYSLIILGLVLSDRGTYSCVVQKKERGTYEVKHLALVKLSIKADFSTPNITESGNPSADTKRITCFASGGFPKPRFSWLENGRELPGINTTISQDPESELYTISSQLDFNTTRNHTIKCLIKYGDAHVSEDFTWEKPPEDPPDSGSGGGGSGGGGSGGGGSAESKYGPPCPPCPAPEAAGGPSVFLFPPKPKDQLMISRTPEVTCVVVDVSQEDPEVQFNWYVDGVEVHNAKTKPREEQFNSTYRVVSVLTVLHQDWLNGKEYKCKVSNKGLPSSIEKTISKAKGQPREPQVYTLPPSQEEMTKNQVSLTCLVKGFYPSDIAVEWESNGQPENNYKTTPPVLDSDGSFFLYSRLTVDKSRWQEGNVFSCSVLHEALHNHYTQKSLSLSLGGGGGSAPTSSSTKKTQLQLEHLLLDLQMILNGINNYKNPKLTAMLTAKFYMPKKATELKHLQCLERELKPLEEVLNLAQSKNFHLRPRDLISNINVIVLELKGSETTFMCEYADETATIVEFLNRWITFCQSIISTLT

SEQ ID NO: 35 - protein, 153 aa, synthetic construct
  REGION 1..153: note = wild type hIL-2
MYRMQLLSCIALSLALVTNSAPTSSSTKKTQLQLEHLLLDLQMILNGINNYKNPKLTRMLTFKFYMPKKATELKHLQCLEEELKPLEEVLNLAQSKNFHLRPRDLISNINVIVLELKGSETTFMCEYADETATIVEFLNRWITFCQSIISTLT

SEQ ID NO: 36 - protein, 158 aa, synthetic construct
  REGION 1..158: note = IL-2 with signal sequence
MDAMLRGLCCVLLLCGAVFVSPSHAAPTSSSTKKTQLQLEHLLLDLQMILNGINNYKNPKLTRMLTFKFYMPKKATELKHLQCLEEELKPLEEVLNLAQSKNFHLRPRDLISNINVIVLELKGSETTFMCEYADETATIVEFLNRWITFCQSIISTLT

SEQ ID NO: 37 - DNA, 474 bp, synthetic construct
  misc_feature 1..474: note = nucleotide sequence coding IL-2 with signal sequence
  source 1..474: mol_type = other DNA
atggatgctatgctgagaggcctgtgttgcgtgctgctgctgtgtggcgctgtgttcgtgtctccttctcacgctgcccctaccagctcctctaccaagaaaacccagctccagttggagcatctgctgctggacctccagatgattctgaacgggatcaacaactataagaaccccaagctgacccgcatgctgacctttaagttctacatgcccaagaaggccaccgagctgaagcacctccagtgcctggaagaagaactgaagcccctggaagaggtgctgaatctggcccagtccaagaacttccacctgaggccacgggacctgatcagcaacatcaacgtgatcgtgctggaactgaagggctccgagacaacctttatgtgcgagtacgccgacgagacagccaccatcgtggaatttctgaaccggtggatcaccttctgccagagcatcatctccacactgacc